European Patent Application EP 4 428 245 A1, published September 11, 2024. Title: A METHOD FOR DETECTING AMYLOID β BOUND TO EXOSOMES DERIVED FROM BRAIN NERVE CELLS IN BLOOD, A KIT FOR DETECTING AMYLOID β BOUND TO EXOSOMES DERIVED FROM BRAIN NERVE CELLS IN BLOOD, AND A METHOD FOR EVALUATING ACCUMULATION LEVEL OF AMYLOID β IN A BRAIN. Applicant: 凸版印刷株式会社. The sequence listing filed with the application follows.

SEQUENCE LISTING (3 sequences)

SEQ ID NO: 1 - DNA, 75 bp, synthetic construct
  misc_feature 1..75: note = synthesized oligonucleotide sequence
  source 1..75: mol_type = other DNA
tttgtcactgttcctccttttgttttcctttctgtgagcaatttcacccaaattggaaccatgctgtatacagtt

SEQ ID NO: 2 - DNA, 28 bp, synthetic construct
  misc_feature 1..28: note = synthesized oligonucleotide sequence
  source 1..28: mol_type = other DNA
cgcgccgaggaattgctcacagaaagga

SEQ ID NO: 3 - DNA, 22 bp, synthetic construct
  misc_feature 1..22: note = synthesized oligonucleotide sequence
  source 1..22: mol_type = other DNA
gcatggttccaatttgggtgat